European Patent Specification EP 3 334 826 B1, published October 11, 2023. Title: HIGH THEBAINE POPPY AND METHODS OF PRODUCING THE SAME. Applicant: API LABS INC. The sequence listing filed with the application follows.

SEQUENCE LISTING (16 sequences)

SEQ ID NO: 1 - protein, 364 aa, Papaver somniferum T6ODM
MEKAKLMKLGNGMEIPSVQELAKLTLAEIPSRYVCANENLLLPMGASVINDHETIPVIDIENLLSPEPIIGKLELDRLHFACKEWGFFQVVNHGVDASLVDSVKSEIQGFFNLSMDEKTKYEQEDGDVEGFGQGFIESEDQTLDWADIFMMFTLPLHLRKPHLFSKLPVPLRETIESYSSEMKKLSMVLFNKMEKALQVQAAEIKGMSEVFIDGTQAMRMNYYPPCPQPNLAIGLTSHSDFGGLTILLQINEVEGLQIKREGTWISVKPLPNAFVVNVGDILEIMTNGIYHSVDHRAVVNSTNERLSIATFHDPSLESVIGPISSLITPETPALFKSGSTYGDLVEECKTRKLDGKSFLDSMRI

SEQ ID NO: 2 - DNA, 1386 bp, Papaver somniferum T6ODM
gttcttaattcattaattaatttagaaaaatcatggagaaagcaaaacttatgaagctaggtaatggtatggaaataccaagtgttcaagaattggctaaactcacgcttgccgaaattccatctcgatacgtatgcgccaatgaaaaccttttgttgcctatgggtgcatctgtcataaatgatcatgaaaccattcctgtcatcgatatagaaaatttattatctccagaaccaataatcggaaagttagaattagataggcttcattttgcttgcaaagaatggggtttttttcaggtagtgaaccatggagtcgacgcttcattggtggatagtgtaaaatcagaaattcaaggtttctttaacctttctatggatgagaaaactaaatatgaacaggaagatggagatgtggaaggatttggacaaggctttattgaatcagaggaccaaacacttgattgggcagatatatttatgatgttcactcttccactccatttaaggaagcctcacttattttcaaaactcccagtgcctctcagggagacaatcgaatcctactcatcagaaatgaaaaagttatccatggttctctttaataagatggaaaaagctctacaagtacaagcagccgagattaagggtatgtcagaggtgtttatagatgggacacaagcaatgaggatgaactattatcccccttgtcctcaaccaaatctcgccatcggtcttacgtcgcactcggattttggcggtttgacaatcctccttcaaatcaacgaagtggaaggattacagataaaaagagaggggacatggatttcagtcaaacctctacctaatgcgttcgtagtgaatgttggagatattttggagataatgactaatggaatttaccatagtgtcgatcaccgggcagtagtaaactcaacaaatgagaggctctcaatcgcaacatttcatgaccctagtctagagtcggtaataggcccaatatcaagcttgattactccagagacacctgctttgtttaaaagtggatctacatatggggatcttgtggaggaatgtaaaacaaggaagctcgatggaaaatcatttcttgactccatgaggatttgaaaactcaagaaaaaataatacgacgtgattgcatgtcagattcaactatccttttgtcgttttttggtgctcgagtccttaattgttttgatcattgcttttgattctaattaataagacttttctcaagaaccacatgtaatgtacctttactttcagaaaataaaaagtattgaggcacaaatgagaaaattgagagagtgcttgagaagtgtaatttctcgaaagtgcgttgtgtttgaaaaaaaaaaaaaaaaaa

SEQ ID NO: 3 - protein, 360 aa, Papaver somniferum CODM
METPILIKLGNGLSIPSVQELAKLTLAEIPSRYTCTGESPLNNIGASVTDDETVPVIDLQNLLSPEPVVGKLELDKLHSACKEWGFFQLVNHGVDALLMDNIKSEIKGFFNLPMNEKTKYGQQDGDFEGFGQPYIESEDQRLDWTEVFSMLSLPLHLRKPHLFPELPLPFRETLESYLSKMKKLSTVVFEMLEKSLQLVEIKGMTDLFEDGLQTMRMNYYPPCPRPELVLGLTSHSDFSGLTILLQLNEVEGLQIRKEERWISIKPLPDAFIVNVGDILEIMTNGIYRSVEHRAVVNSTKERLSIATFHDSKLESEIGPISSLVTPETPALFKRGRYEDILKENLSRKLDGKSFLDYMRM

SEQ ID NO: 4 - DNA, 1452 bp, Papaver somniferum CODM
gtaaagattgatatatgatctgaagatctgacaagaaagttcatcaaatatagagttcatggagacaccaatacttatcaagctaggcaatggtttgtcaataccaagtgttcaggaattggctaaactcacgcttgcagaaattccatctcgatacacatgcaccggtgaaagcccgttgaataatattggtgcgtctgtaacagatgatgaaacagttcctgtcatcgatttgcaaaatttactatctccagaacccgtagttggaaagttagaattggataagcttcattctgcttgcaaagaatggggtttctttcagctggttaaccatggagtcgacgctttactgatggacaatataaaatcagaaattaaaggtttctttaaccttccaatgaatgagaaaactaaatacggacagcaagatggagattttgaaggatttggacaaccctatattgaatcggaggaccaaagacttgattggactgaagtgtttagcatgttaagtcttcctctccatttaaggaagcctcatttgtttccagaactccctctgcctttcagggagacactggaatcctacctatcaaaaatgaaaaaactatcaacggttgtctttgagatgttggaaaaatctctacaattagttgagattaaaggtatgacagacttatttgaagatgggttgcaaacaatgaggatgaactattatcctccttgtcctcgaccagagcttgtacttggtcttacgtcacactcggattttagcggtttgacaattctccttcaacttaatgaagttgaaggattacaaataagaaaagaagagaggtggatttcaatcaaacctctacctgatgcgttcatagtgaatgttggagacattttggagataatgactaatgggatttaccgtagcgtcgagcaccgggcagtagtaaactcaacaaaggagaggctctcaatcgcgacatttcatgactctaaactagagtcagaaataggcccaatttcgagcttggtcacaccagagacacctgctttgttcaaaagaggtaggtatgaggatattttgaaggaaaatctttcaaggaagcttgatggaaaatcatttctcgactacatgaggatgtgagaaagtgtgaacatatattatactccacattgtgtttaatatatgatgaaataagttgcttttgaagtatgatgaaataagttggttttgaagaattcatattgtgcttaaatttcgtggatgactgagagatttattatgtaataataatgtattggtttgaagattctcgtctcactatatgtaagactctgtttgggtcaagtgatgtaatcacggttgaaataagttgcttttgaagaattcatatggtgcttaatattatgtaataaataatgtattggattgaaaaaaaaaaaaaaaaaaaaaaa

SEQ ID NO: 5 - DNA, 8688 bp, Artificial Sequence
  TDNA sequence
tcctgtggttggcatgcacatacaaatggacgaacggataaaccttttcacgcccttttaaatatccgattattctaataaacgctcttttctcttaggtttacccgccaatatatcctgtcaaacactgatagtttaaactgaaggcgggaaacgacaatctgctagtggatctcccagtcacgacgttgtaaaacgggcgccccgcggaaagcttgctagccaattggggcccaacgttctcgagaacgtggatacttggcagtggttacttggcttttcctttattttcttttggacggaagcggtggttactttgtcacacatttaaaaaaacacgtgtttctcacttttttctattcccgtcacaaacaattttaagaaagatccatctatcgtgatctttctatcaaacaaaagaaaaaaggtcttcatagtaacgctacaacatcaaatatgtggttgctctgacatcagtcgggaaaataaggatatggcggcattggccacatctattggggtcccaacttcctttcacaaaaaaattaaattgggtgtcccaacttttatctttgatatagtgacatgagtatcgggagcattggacaatggataaaatgagaactaaaaaaattctggttaatttttgatcattgttatttaaaaggttattttatctataatctacccatattgatcagttttatttaaatttgtttagctaccgctccacgagagagatcctcatcttaaaaatggaatatggaaattacacacgaccccaaaagtatattttttctctggagaatgctatttagagctttgactatatggtctgaattagaaagacgggaaataaaatctgctaagtgatataagctctaagtaggcgatgtgtgatggagaacaccttttctttaacagtcttcatgttttacagattcgcgaacttcgaatatccctatacggtctgtctaaccctcgtgtgtcttttgagtccaagataaaggccattattgagtaacatagacatgctggaatccaaccattgaagtcacaactgtccatgtagattctttggagaatctgaaaagtcttaataaaggtggtgtttcaaagaaaacaaaacaaatgagttaagaaaaaaaaatatcatgtagtggtcgagtattatgttatttattgtgtagctaccaatctttattctttaaatctgacataaaatgctacaaactttttacctcgtctatagccccaaaaaacctaaccacggttctaaaaccacacacagtgattttggttgacgacaatgcctctccttcctcaaaacgatttatttacattttttaaatcaaatgttacattttataccataattaagtctttttacagaatacttagatggaagagatgtataaaaaaggaggaaattgtaaaaaacatatttcgatcaattaaaccaggattcataaaaatataagtatatatataaatgatgtttcgtttagcgatgaacttcactcatatgataatacttaacaatataagtacataaaaaataaaataaaattaattgtttacgaaaagtctacaaatactgcatgtataattaatgttctctttatttatttatttataccttaccaagatatatctataaccgcatagaaatagaaggcgaagagataatttccaaaaacaagaaaaacctctaagctcaaaagtctagaaggccttggatccacccatggaggttgtcacagtatcacttgtagcagttgtgatcactactttcttatacttaatcttcagagattcaagtcctaaaggtttgccaccaggtccaaaaccctggccaatagttggaaaccttcttcaacttggtgagaaacctcattctcagtttgctcagcttgctgaaacctatggtgatctcttttcactgaaactaggaagtgaaacggttgttgtagcttcaactccattagcagctagcgagattctaaagacgcatgatcgtgttctctctggtcgatacgtgtttcaaagtttccgggtaaaggaacatgtggagaactctattgtgtggtctgaatgtaatgaaacatggaagaaactgcggaaagtttgtagaacggaactttttacgcagaagatgattgaaagtcaagctgaagttagagaaagtaaggctatggaaatggtggagtatttgaagaaaaatgtaggaaatgaagtgaaaattgctgaagttgtatttgggacgttggtgaatatattcggtaacttgatattttcacaaaatattttcaagttgggtgatgaaagtagtggaagtgtagaaatgaaagaacatctatggagaatgctggaattggggaactcgacaaatccagctgattattttccatttttgggtaaattcgatttgtttggacaaagaaaagatgttgctgattgtctgcaagggatttatagtgtttggggtgctatgctcaaagaaagaaaaatagccaagcagcataacaacagcaagaagaatgattttgttgagattttgctcgattccggactcgatgaccagcagattaatgccttgctcatggaaatatttggtgcgggaacagagacaagtgcatctacaatagaatgggcgttgtctgagctcacaaaaaaccctcaagtaacagccaatatgcggttggaattgttatctgtggtagggaagaggccggttaaggaatccgacataccaaacatgccttatcttcaagcttttgttaaagaaactctacggcttcatccagcaactcctctgctgcttccacgtcgagcacttgagacctgcaaagttttgaactatacgatcccgaaagagtgtcagattatggtgaacgcctggggcattggtcgggatccaaaaaggtggactgatccattgaagttttcaccagagaggttcttgaattcgagcattgatttcaaagggaacgacttcgagttgataccatttggtgcagggagaaggatatgtcctggtgtgcccttggcaactcaatttattagtcttattgtgtctagtttggtacagaattttgattggggattaccgaagggaatggatcctagccaactgatcatggaagagaaatttgggtgacactgcaaaaggaaccacctctgtatattgttcctaaaactcgggattaagggagaattcgtcgactttgcggccgcatcgatactgcaggagctcggtaccttttactagtgatatccctgtgtgaaattgttatccgctacgcgtgatcgttcaaacatttggcaataaagtttcttaagattgaatcctgttgccggtcttgcgatgattatcatataatttctgttgaattacgttaagcatgtaataattaacatgtaatgcatgacgttatttatgagatgggtttttatgattagagtcccgcaattatacatttaatacgcgatagaaaacaaaatatagcgcgcaaactaggataaattatcgcgcgcggtgtcatctatgttactagatcccatgggaagttcctattccgaagttcctattctctgaaaagtataggaacttcagcgatcgctccaatcccacaaaaatctgagcttaacagcacagttgctcctctcagagcagaatcgggtattcaacaccctcatatcaactactacgttgtgtataacggtccacatgccggtatatacgatgactggggttgtacaaaggcggcaacaaacggcgttcccggagttgcacacaagaaatttgccactattacagaggcaagagcagcagctgacgcgtacacaacaagtcagcaaacagacaggttgaacttcatccccaaaggagaagctcaactcaagcccaagagctttgctaaggccctaacaagcccaccaaagcaaaaagcccactggctcacgctaggaaccaaaaggcccagcagtgatccagccccaaaagagactcctttgccccggagattacaatggacgatttcctctatctttacgatctaggaaggaagttcgaaggtgaaggtgacgacactatgttcaccactgataatgagaaggttagcctcttcaatttcagaaagaatgctgacccacagatggttagagaggcctacgcagcaggtctcatcaagacgatctacccgagtaacaatctccaggagatcaaataccttcccaagaaggttaaagatgcagtcaaaagattcaggactaattgcatcaagaacacagagaaagacatatttctcaagatcagaagtactattccagtatggacgattcaaggcttgcttcataaaccaaggcaagtaatagagattggagtctctaaaaaggtagttcctactgaatctaaggccatgcatggagtctaagattcaaatcgaggatctaacagaactcgccgtgaagactggcgaacagttcatacagagtcttttacgactcaatgacaagaagaaaatcttcgtcaacatggtggagcacgacactctggtctactccaaaaatgtcaaagatacagtctcagaagaccaaagggctattgagacttttcaacaaaggataatttcgggaaacctcctcggattccattgcccagctatctgtcacttcatcgaaaggacagtagaaaaggaaggtggctcctacaaatgccatcattgcgataaaggaaaggctatcattcaagatctctctgccgacagtggtcccaaagatggacccccacccacgaggagcatcgtggaaaaagaagacgttccaaccacgtcttcaaagcaagtggattgatgtgacatctccactgacgtaagggatgacgcacaatcccactatccttcgcaagacccttcctctatataaggaagttcatttcatttggagaggacacgctcgagtataagagctctatttttacaacaattaccaacaacaacaaacaacaaacaacattacaattacatttacaattaccatggggcgcgccccttgtcctcaaccaaatctcgccatcggtcttacgtcgcactcggattttggcggtttgacaatcctccttcaaatcaacgaagtggaaggattacagataaaaagagaggggacatggatttcagtcaaacctctacctaatgcgttcgtagtgaatgttggagatattttggagataatgactaatggaatttaccatagtgtcgatcaccgggcagtagtaaactcaacaaatgagaggctctcaatcgcaacatttcatgaccctagtctagagtcggtaataggcccaatatcaagcttgattactccagagacacctgctttgtttaaaagtggaatttaaatccccagatgaacatggcatcgtggtgattgatgaaactgctgctgtcggctttaacctctctttaggcattggtttcgaagcgggcaacaagccgaaagaactgtacagcgaagaggcagtcaacggggaaactcagcaagcgcacttacaggcgattaaagagctgatagcgcgtgacaaaaaccacccaagcgtggtgatgtggagtattgccaacgaaccggatacccgtccgcaaggtgcacgggaatatttcgcgccactggcggaagcaacgcgtaaactcgacccgacgcgtccgatcacctgcgtcaatgtaatgttctgcgacgctcacaccgataccatcagcgatctctttgatggggatcctccacttttaaacaaagcaggtgtctctggagtaatcaagcttgatattgggcctattaccgactctagactagggtcatgaaatgttgcgattgagagcctctcatttgttgagtttactactgcccggtgatcgacactatggtaaattccattagtcattatctccaaaatatctccaacattcactacgaacgcattaggtagaggtttgactgaaatccatgtcccctctctttttatctgtaatccttccacttcgttgatttgaaggaggattgtcaaaccgccaaaatccgagtgcgacgtaagaccgatggcgagatttggttgaggacaaggactagtccctagagtcctgctttaatgagatatgcgagacgcctatgatcgcatgatatttgctttcaattctgttgtgcacgttgtaaaaaacctgagcatgtgtagctcagatccttaccgccggtttcggttcattctaatgaatgaatatatcacccgttactatcgtatttttatgaataatattctccgttcaatttactgattgtaccctactacttatatgtacaatattaaaatgaaaacaatatattgtgctgaataggtttatagcgacatctatgatagagcgccacaataacaaacaattgcgttttattattacaaatccaattttaaaaaaagcggcagaaccggtcaaacctaaaagactgattacataaatcttattcaaatttcaaaagtgccccaggggctagtatctacgacacaccgagcggcgaactaataacgctcactgaagggaactccggttccccgccggcgcgcatgggtgagattccttgaagttgagtattggccgtccgctctaccgaaagttacgggcaccattcaacccggtccagcacggcggccgggtaaccgacttgctgccccgagaattatgcagcatttttttggtgtatgtgggccccaaatgaagtgcaggtcaaaccttgacagtgacgacaaatcgttgggcgggtccagggcgaattttgcgacaacatgtcgaggctcagcagggcgatcgcagacgtcgggatcttctgcaagcatctctatttcctgaaggtctaacctcgaagatttaagatttaattacgtttataattacaaaattgattctagtatctttaatttaatgcttatacattattaattaatttagtactttcaatttgttttcagaaattattttactattttttataaaataaaagggagaaaatggctatttaaatactagcctattttatttcaattttagcttaaaatcagccccaattagccccaatttcaaattcaaatggtccagcccaattcctaaataacccacccctaacccgcccggtttccccttttgatccatgcagtcaacgcccagaatttccctatataattttttaattcccaaacacccctaactctatcccatttctcaccaaccgccacatagatctatcctcttatctctcaaactctctcgaaccttcccctaaccctagcagcctctcatcatcctcacctcaaaacccaccggggccggccatgattgaacaagatggattgcacgcaggttctccggccgcttgggtggagaggctattcggctatgactgggcacaacagacaatcggctgctctgatgccgccgtgttccggctgtcagcgcaggggaggccggttctttttgtcaagaccgacctgtccggtgccctgaatgaacttcaagacgaggcagcgcggctatcgtggctggccacgacgggcgttccttgcgcagctgtgctcgacgttgtcactgaagcgggaagggactggctgctattgggcgaagtgccggggcaggatctcctgtcatctcaccttgctcctgccgagaaagtatccatcatggctgatgcaatgcggcggctgcatacgcttgatccggctacctgcccattcgaccaccaagcgaaacatcgcatcgagcgagcacgtactcggatggaagccggtcttgtcgatcaggatgatctggacgaagagcatcaggggctcgcgccagccgaactgttcgccaggctcaaggcgcgcatgcccgacggcgaggatctcgtcgtgactcatggcgatgcctgcttgccgaatatcatggtggaaaatggccgcttttctggattcatcgactgtggccggctgggtgtggcggaccgctatcaggacatagcgttggctacccgtgatattgctgaagagcttggcggcgaatgggctgaccgcttcctcgtgctttacggtatcgccgctcccgattcgcagcgcatcgccttctatcgccttcttgacgagttcttctgaggcgcgccgatcgttcaaacatttggcaataaagtttcttaagattgaatcctgttgccggtcttgcgatgattatcatataatttctgttgaattacgttaagcatgtaataattaacatgtaatgcatgacgttatttatgagatgggtttttatgattagagtcccgcaattatacatttaatacgcgatagaaaacaaaatatagcgcgcaaactaggataaattatcgcgcgcggtgtcatctatgttactagatccctagggaagttcctattccgaagttcctattctctgaaaagtataggaacttctttgcgtattgggcgctcttggcctttttggccaccggtcgtacggttaaaaccaccccagtacattaaaaacgtccgcaatgtgttattaagttgtctaagcgtcaatttgtttacaccacaatatatcctgccaccagccagccaacagctccccgaccggcagctcggcacaaaatcaccactcgatacaggcagcccatcagtcc

SEQ ID NO: 6 - DNA, 3238 bp, Artificial Sequence
  expression cassette including promoter
gcgatcgctccaatcccacaaaaatctgagcttaacagcacagttgctcctctcagagcagaatcgggtattcaacaccctcatatcaactactacgttgtgtataacggtccacatgccggtatatacgatgactggggttgtacaaaggcggcaacaaacggcgttcccggagttgcacacaagaaatttgccactattacagaggcaagagcagcagctgacgcgtacacaacaagtcagcaaacagacaggttgaacttcatccccaaaggagaagctcaactcaagcccaagagctttgctaaggccctaacaagcccaccaaagcaaaaagcccactggctcacgctaggaaccaaaaggcccagcagtgatccagccccaaaagagactcctttgccccggagattacaatggacgatttcctctatctttacgatctaggaaggaagttcgaaggtgaaggtgacgacactatgttcaccactgataatgagaaggttagcctcttcaatttcagaaagaatgctgacccacagatggttagagaggcctacgcagcaggtctcatcaagacgatctacccgagtaacaatctccaggagatcaaataccttcccaagaaggttaaagatgcagtcaaaagattcaggactaattgcatcaagaacacagagaaagacatatttctcaagatcagaagtactattccagtatggacgattcaaggcttgcttcataaaccaaggcaagtaatagagattggagtctctaaaaaggtagttcctactgaatctaaggccatgcatggagtctaagattcaaatcgaggatctaacagaactcgccgtgaagactggcgaacagttcatacagagtcttttacgactcaatgacaagaagaaaatcttcgtcaacatggtggagcacgacactctggtctactccaaaaatgtcaaagatacagtctcagaagaccaaagggctattgagacttttcaacaaaggataatttcgggaaacctcctcggattccattgcccagctatctgtcacttcatcgaaaggacagtagaaaaggaaggtggctcctacaaatgccatcattgcgataaaggaaaggctatcattcaagatctctctgccgacagtggtcccaaagatggacccccacccacgaggagcatcgtggaaaaagaagacgttccaaccacgtcttcaaagcaagtggattgatgtgacatctccactgacgtaagggatgacgcacaatcccactatccttcgcaagacccttcctctatataaggaagttcatttcatttggagaggacacgctcgagtataagagctctatttttacaacaattaccaacaacaacaaacaacaaacaacattacaattacatttacaattaccatggggcgcgccccttgtcctcaaccaaatctcgccatcggtcttacgtcgcactcggattttggcggtttgacaatcctccttcaaatcaacgaagtggaaggattacagataaaaagagaggggacatggatttcagtcaaacctctacctaatgcgttcgtagtgaatgttggagatattttggagataatgactaatggaatttaccatagtgtcgatcaccgggcagtagtaaactcaacaaatgagaggctctcaatcgcaacatttcatgaccctagtctagagtcggtaataggcccaatatcaagcttgattactccagagacacctgctttgtttaaaagtggaatttaaatccccagatgaacatggcatcgtggtgattgatgaaactgctgctgtcggctttaacctctctttaggcattggtttcgaagcgggcaacaagccgaaagaactgtacagcgaagaggcagtcaacggggaaactcagcaagcgcacttacaggcgattaaagagctgatagcgcgtgacaaaaaccacccaagcgtggtgatgtggagtattgccaacgaaccggatacccgtccgcaaggtgcacgggaatatttcgcgccactggcggaagcaacgcgtaaactcgacccgacgcgtccgatcacctgcgtcaatgtaatgttctgcgacgctcacaccgataccatcagcgatctctttgatggggatcctccacttttaaacaaagcaggtgtctctggagtaatcaagcttgatattgggcctattaccgactctagactagggtcatgaaatgttgcgattgagagcctctcatttgttgagtttactactgcccggtgatcgacactatggtaaattccattagtcattatctccaaaatatctccaacattcactacgaacgcattaggtagaggtttgactgaaatccatgtcccctctctttttatctgtaatccttccacttcgttgatttgaaggaggattgtcaaaccgccaaaatccgagtgcgacgtaagaccgatggcgagatttggttgaggacaaggactagtccctagagtcctgctttaatgagatatgcgagacgcctatgatcgcatgatatttgctttcaattctgttgtgcacgttgtaaaaaacctgagcatgtgtagctcagatccttaccgccggtttcggttcattctaatgaatgaatatatcacccgttactatcgtatttttatgaataatattctccgttcaatttactgattgtaccctactacttatatgtacaatattaaaatgaaaacaatatattgtgctgaataggtttatagcgacatctatgatagagcgccacaataacaaacaattgcgttttattattacaaatccaattttaaaaaaagcggcagaaccggtcaaacctaaaagactgattacataaatcttattcaaatttcaaaagtgccccaggggctagtatctacgacacaccgagcggcgaactaataacgctcactgaagggaactccggttccccgccggcgcgcatgggtgagattccttgaagttgagtattggccgtccgctctaccgaaagttacgggcaccattcaacccggtccagcacggcggccgggtaaccgacttgctgccccgagaattatgcagcatttttttggtgtatgtgggccccaaatgaagtgcaggtcaaaccttgacagtgacgacaaatcgttgggcgggtccagggcgaattttgcgacaacatgtcgaggctcagcagggcgatcgca

SEQ ID NO: 7 - DNA, 1067 bp, Artificial Sequence
  hairpin construct
ccccttgtcctcaaccaaatctcgccatcggtcttacgtcgcactcggattttggcggtttgacaatcctccttcaaatcaacgaagtggaaggattacagataaaaagagaggggacatggatttcagtcaaacctctacctaatgcgttcgtagtgaatgttggagatattttggagataatgactaatggaatttaccatagtgtcgatcaccgggcagtagtaaactcaacaaatgagaggctctcaatcgcaacatttcatgaccctagtctagagtcggtaataggcccaatatcaagcttgattactccagagacacctgctttgtttaaaagtggaatttaaatccccagatgaacatggcatcgtggtgattgatgaaactgctgctgtcggctttaacctctctttaggcattggtttcgaagcgggcaacaagccgaaagaactgtacagcgaagaggcagtcaacggggaaactcagcaagcgcacttacaggcgattaaagagctgatagcgcgtgacaaaaaccacccaagcgtggtgatgtggagtattgccaacgaaccggatacccgtccgcaaggtgcacgggaatatttcgcgccactggcggaagcaacgcgtaaactcgacccgacgcgtccgatcacctgcgtcaatgtaatgttctgcgacgctcacaccgataccatcagcgatctctttgatggggatcctccacttttaaacaaagcaggtgtctctggagtaatcaagcttgatattgggcctattaccgactctagactagggtcatgaaatgttgcgattgagagcctctcatttgttgagtttactactgcccggtgatcgacactatggtaaattccattagtcattatctccaaaatatctccaacattcactacgaacgcattaggtagaggtttgactgaaatccatgtcccctctctttttatctgtaatccttccacttcgttgatttgaaggaggattgtcaaaccgccaaaatccgagtgcgacgtaagaccgatggcgagatttggttgaggacaagg

SEQ ID NO: 8 - DNA, 342 bp, Artificial Sequence
  sense strand of hairpin construct
ccttgtcctcaaccaaatctcgccatcggtcttacgtcgcactcggattttggcggtttgacaatcctccttcaaatcaacgaagtggaaggattacagataaaaagagaggggacatggatttcagtcaaacctctacctaatgcgttcgtagtgaatgttggagatattttggagataatgactaatggaatttaccatagtgtcgatcaccgggcagtagtaaactcaacaaatgagaggctctcaatcgcaacatttcatgaccctagtctagagtcggtaataggcccaatatcaagcttgattactccagagacacctgctttgtttaaaagtgga

SEQ ID NO: 9 - DNA, 20 bp, Artificial Sequence
  Synthetic primer
taaccgacttgctgccccga

SEQ ID NO: 10 - DNA, 27 bp, Artificial Sequence
  Synthetic primer
aaatagagatgcttgcagaagatcccg

SEQ ID NO: 11 - DNA, 24 bp, Artificial Sequence
  Synthetic primer
cgtttgaatcttgctggccgtgat

SEQ ID NO: 12 - DNA, 24 bp, Artificial Sequence
  Synthetic primer
tagacgagctgcctttggaagtgt

SEQ ID NO: 13 - DNA, 21 bp, Artificial Sequence
  Synthetic primer
cgtcttgcgcactgatttgaa

SEQ ID NO: 14 - DNA, 24 bp, Artificial Sequence
  Synthetic primer
cgtttgaatcttgctggccgtgat

SEQ ID NO: 15 - DNA, 1386 bp, Artificial Sequence
  T6ODM RNA transcript
guucuuaauucauuaauuaauuuagaaaaaucauggagaaagcaaaacuuaugaagcuagguaaugguauggaaauaccaaguguucaagaauuggcuaaacucacgcuugccgaaauuccaucucgauacguaugcgccaaugaaaaccuuuuguugccuaugggugcaucugucauaaaugaucaugaaaccauuccugucaucgauauagaaaauuuauuaucuccagaaccaauaaucggaaaguuagaauuagauaggcuucauuuugcuugcaaagaaugggguuuuuuucagguagugaaccauggagucgacgcuucauugguggauaguguaaaaucagaaauucaagguuucuuuaaccuuucuauggaugagaaaacuaaauaugaacaggaagauggagauguggaaggauuuggacaaggcuuuauugaaucagaggaccaaacacuugauugggcagauauauuuaugauguucacucuuccacuccauuuaaggaagccucacuuauuuucaaaacucccagugccucucagggagacaaucgaauccuacucaucagaaaugaaaaaguuauccaugguucucuuuaauaagauggaaaaagcucuacaaguacaagcagccgagauuaaggguaugucagagguguuuauagaugggacacaagcaaugaggaugaacuauuaucccccuuguccucaaccaaaucucgccaucggucuuacgucgcacucggauuuuggcgguuugacaauccuccuucaaaucaacgaaguggaaggauuacagauaaaaagagaggggacauggauuucagucaaaccucuaccuaaugcguucguagugaauguuggagauauuuuggagauaaugacuaauggaauuuaccauagugucgaucaccgggcaguaguaaacucaacaaaugagaggcucucaaucgcaacauuucaugacccuagucuagagucgguaauaggcccaauaucaagcuugauuacuccagagacaccugcuuuguuuaaaaguggaucuacauauggggaucuuguggaggaauguaaaacaaggaagcucgauggaaaaucauuucuugacuccaugaggauuugaaaacucaagaaaaaauaauacgacgugauugcaugucagauucaacuauccuuuugucguuuuuuggugcucgaguccuuaauuguuuugaucauugcuuuugauucuaauuaauaagacuuuucucaagaaccacauguaauguaccuuuacuuucagaaaauaaaaaguauugaggcacaaaugagaaaauugagagagugcuugagaaguguaauuucucgaaagugcguuguguuugaaaaaaaaaaaaaaaaaa

SEQ ID NO: 16 - RNA, 1452 nt, Artificial Sequence
  CODM RNA transcript
guaaagauugauauaugaucugaagaucugacaagaaaguucaucaaauauagaguucauggagacaccaauacuuaucaagcuaggcaaugguuugucaauaccaaguguucaggaauuggcuaaacucacgcuugcagaaauuccaucucgauacacaugcaccggugaaagcccguugaauaauauuggugcgucuguaacagaugaugaaacaguuccugucaucgauuugcaaaauuuacuaucuccagaacccguaguuggaaaguuagaauuggauaagcuucauucugcuugcaaagaaugggguuucuuucagcugguuaaccauggagucgacgcuuuacugauggacaauauaaaaucagaaauuaaagguuucuuuaaccuuccaaugaaugagaaaacuaaauacggacagcaagauggagauuuugaaggauuuggacaacccuauauugaaucggaggaccaaagacuugauuggacugaaguguuuagcauguuaagucuuccucuccauuuaaggaagccucauuuguuuccagaacucccucugccuuucagggagacacuggaauccuaccuaucaaaaaugaaaaaacuaucaacgguugucuuugagauguuggaaaaaucucuacaauuaguugagauuaaagguaugacagacuuauuugaagauggguugcaaacaaugaggaugaacuauuauccuccuuguccucgaccagagcuuguacuuggucuuacgucacacucggauuuuagcgguuugacaauucuccuucaacuuaaugaaguugaaggauuacaaauaagaaaagaagagagguggauuucaaucaaaccucuaccugaugcguucauagugaauguuggagacauuuuggagauaaugacuaaugggauuuaccguagcgucgagcaccgggcaguaguaaacucaacaaaggagaggcucucaaucgcgacauuucaugacucuaaacuagagucagaaauaggcccaauuucgagcuuggucacaccagagacaccugcuuuguucaaaagagguagguaugaggauauuuugaaggaaaaucuuucaaggaagcuugauggaaaaucauuucucgacuacaugaggaugugagaaagugugaacauauauuauacuccacauuguguuuaauauaugaugaaauaaguugcuuuugaaguaugaugaaauaaguugguuuugaagaauucauauugugcuuaaauuucguggaugacugagagauuuauuauguaauaauaauguauugguuugaagauucucgucucacuauauguaagacucuguuugggucaagugauguaaucacgguugaaauaaguugcuuuugaagaauucauauggugcuuaauauuauguaauaaauaauguauuggauugaaaaaaaaaaaaaaaaaaaaaaa